European Patent Specification EP 4 046 624 B1, published September 3, 2025. Title: USES OF WHITE ROSELLE EXTRACT FOR SKIN HYDRATING. Applicant: TCI CO., LTD. The sequence listing filed with the application follows.

SEQUENCE LISTING (18 sequences)

SEQ ID NO: 1 - DNA, 22 bp, Artificial Sequence
  TGM1
gatcgcatcacccttgagttac

SEQ ID NO: 2 - DNA, 19 bp, Artificial Sequence
  TGM1
gcaggttcagattctgccc

SEQ ID NO: 3 - DNA, 21 bp, Artificial Sequence
  KRT1
agagtggaccaactgaagagt

SEQ ID NO: 4 - DNA, 21 bp, Artificial Sequence
  KRT1
attctctgcatttgtccgctt

SEQ ID NO: 5 - DNA, 22 bp, Artificial Sequence
  KRT10
tcctacttggacaaagttcggg

SEQ ID NO: 6 - DNA, 19 bp, Artificial Sequence
  KRT10
cccctgatgtgagttgcca

SEQ ID NO: 7 - DNA, 20 bp, Artificial Sequence
  KRT14
ttctgaacgagatgcgtgac

SEQ ID NO: 8 - DNA, 20 bp, Artificial Sequence
  KRT14
gcagctcaatctccaggttc

SEQ ID NO: 9 - DNA, 19 bp, Artificial Sequence
  AQP3
ggggagatgctccacatcc

SEQ ID NO: 10 - DNA, 21 bp, Artificial Sequence
  AQP3
aaaggccaggttgatggtgag

SEQ ID NO: 11 - DNA, 20 bp, Artificial Sequence
  SMPD1
ctgactctcgggttctctgg

SEQ ID NO: 12 - DNA, 20 bp, Artificial Sequence
  SMPD1
tccaccatgtcatcctcaaa

SEQ ID NO: 13 - DNA, 20 bp, Artificial Sequence
  GBA
tccagttgcacaacttcagc

SEQ ID NO: 14 - DNA, 20 bp, Artificial Sequence
  GBA
ttgtgctcagcataggcatc

SEQ ID NO: 15 - DNA, 23 bp, Artificial Sequence
  HAS2
aagaacaacttccacgaaaaggg

SEQ ID NO: 16 - DNA, 20 bp, Artificial Sequence
  HAS2
ggctgggtcaagcatagtgt

SEQ ID NO: 17 - DNA, 19 bp, Artificial Sequence
  HAS3
cgcagcaacttccatgagg

SEQ ID NO: 18 - DNA, 21 bp, Artificial Sequence
  HAS3
agtcgcacacctggatgtagt